European Patent Specification EP 3 365 355 B1, published January 28, 2026. Title: A method for regulating cancer stem cell growth by inhibiting phosphorylation of 120th threonine residue of TSPYL5 protein, a composition containing the peptide sequence functioning to inhibit the phosphorylation and a use thereof. Applicant: Korea Atomic Energy Research Institute Kim, In Gyu Kim, Seo Yeon Lee, Jei Ha Choi, Soo Im Kim, Min Sik Kim, Jung Yul Shin, Byungchul Jung, Uhee. The sequence listing filed with the application follows.

SEQUENCE LISTING (45 sequences)

SEQ ID NO: 1 - DNA, 27 bp, Artificial
  TSPYL5_primer F
cttaagcttatgagcggccgaagtcgg

SEQ ID NO: 2 - DNA, 28 bp, Artificial
  TSPYL5_primer R
tggaattcgtgttggattggctcacccc

SEQ ID NO: 3 - DNA, 29 bp, Artificial
  PTEN_primer R
atataagcttatgacagccatcatcaaag

SEQ ID NO: 4 - DNA, 33 bp, Artificial
  PTEN_primer R
atatgaattctcagactttgtaatttgtgtatg

SEQ ID NO: 5 - DNA, 19 bp, Artificial
  AKT1_primer F
atgagcgacgtggctattg

SEQ ID NO: 6 - DNA, 20 bp, Artificial
  AKT1_primer R
tcaggccgtgccgctggccg

SEQ ID NO: 7 - DNA, 38 bp, Artificial
  T120A_primer F
gagcgcctggccgcagacgctgtcttcgtgggaacagc

SEQ ID NO: 8 - DNA, 38 bp, Artificial
  T120A_primer R
gctgttcccacgaagacagcgtctgcggccaggcgctc

SEQ ID NO: 9 - DNA, 38 bp, Artificial
  T120D_primer F
gagcgcctggccgcagaccatgtcttcgtgggaacagc

SEQ ID NO: 10 - DNA, 38 bp, Artificial
  T120D_primer R
gctgttcccacgaagacatcgtctgcggccaggcgctc

SEQ ID NO: 11 - DNA, 33 bp, Artificial
  T177A_primer F
ggcggcaggggagaatgcctcggtgtcagctgg

SEQ ID NO: 12 - DNA, 33 bp, Artificial
  T177A_primer R
ccagctgacaccgaggcattctcccctgccgcc

SEQ ID NO: 13 - DNA, 34 bp, Artificial
  T326A_primer F
ggtggtgtctcgttctgctccaatccagtggctc

SEQ ID NO: 14 - DNA, 34 bp, Artificial
  T326A_primer R
gagccactggattggagcagaacgagacaccacc

SEQ ID NO: 15 - DNA, 33 bp, Artificial
  T409A_primer F
gcagccaatggagactgctcagcctggggtgag

SEQ ID NO: 16 - DNA, 32 bp, Artificial
  T409A_primer R
tcaccccaggctgagcagtctccattggctgc

SEQ ID NO: 17 - RNA, 25 nt, Artificial
  TSPYL5_primer F1
aaagguagaacugcaagggauuggg

SEQ ID NO: 18 - RNA, 25 nt, Artificial
  TSPYL5_primer R1
cccaaucccuugcaguucuaccuuu

SEQ ID NO: 19 - RNA, 19 nt, Artificial
  PTEN_primer F1
gauaucaagaggauggauu

SEQ ID NO: 20 - RNA, 19 nt, Artificial
  PTEN_primer R1
aauccauccucuugauauc

SEQ ID NO: 21 - RNA, 19 nt, Artificial
  AKT_primer F
gacugacaccagguauuuu

SEQ ID NO: 22 - RNA, 18 nt, Artificial
  AKT_primer R
aaauaccuggugucaguc

SEQ ID NO: 23 - DNA, 21 bp, Artificial
  PTEN_primer F2
cgaactggtgtaatgatatgt

SEQ ID NO: 24 - DNA, 19 bp, Artificial
  PTEN_primer R2
catgaacttgtcttcccgg

SEQ ID NO: 25 - DNA, 20 bp, Artificial
  ALDH1A1_primer F
tgttagctgatgccgacttg

SEQ ID NO: 26 - DNA, 20 bp, Artificial
  ALDH1A1_primer R
ttcttagcccgctcaacact

SEQ ID NO: 27 - DNA, 20 bp, Artificial
  ALDH1A3_primer F
tctcgacaaagccctgaagt

SEQ ID NO: 28 - DNA, 20 bp, Artificial
  ALDH1A3_primer R
tattcggccaaagcgtattc

SEQ ID NO: 29 - DNA, 24 bp, Artificial
  CD44_primer F
atggacaagttttggtggcacgca

SEQ ID NO: 30 - DNA, 24 bp, Artificial
  CD44_primer R
tcaccccaatcttcatgtccacat

SEQ ID NO: 31 - DNA, 20 bp, Artificial
  TSPYL5_primer F2
ttcggctctccaggaagttt

SEQ ID NO: 32 - DNA, 20 bp, Artificial
  TSPYL5_primer R2
ggggatggttctgaaatgct

SEQ ID NO: 33 - DNA, 20 bp, Artificial
  GAPDH_primer F
aagggtcatcatctctgccc

SEQ ID NO: 34 - DNA, 20 bp, Artificial
  GAPDH_primer R
aggggtgctaagcagttggt

SEQ ID NO: 35 - DNA, 23 bp, Artificial
  pALDH1A1_primer F
atttagggcttctgagatcacag

SEQ ID NO: 36 - DNA, 24 bp, Artificial
  pALDH1A1_primer R
acttctcatgctttttaatgctac

SEQ ID NO: 37 - DNA, 23 bp, Artificial
  pALDH1A3_primer F
gcctcagctgtgcactccaggcc

SEQ ID NO: 38 - DNA, 24 bp, Artificial
  pALDH1A3_primer R
tggaacaaagaccggaggcacgga

SEQ ID NO: 39 - DNA, 24 bp, Artificial
  pCD44_primer F
aatgatggatgagaagttgtatgg

SEQ ID NO: 40 - DNA, 24 bp, Artificial
  pCD44_primer R
gatagggctggcatttggctcagc

SEQ ID NO: 41 - DNA, 24 bp, Artificial
  pPTEN_primer F
tttgggcccttgaaattcaacggc

SEQ ID NO: 42 - DNA, 24 bp, Artificial
  pPTEN_primer R
gactgcattcgctctttccttttg

SEQ ID NO: 43 - protein, 15 aa, Artificial
  TS120T
SERLAADTVFVGTAG

SEQ ID NO: 44 - protein, 15 aa, Artificial
  TS120D
SERLAADDVFVGTAG

SEQ ID NO: 45 - protein, 15 aa, Artificial
  TS120A
SERSAADAVFVGTAG